European Patent Application EP 4 545 561 A1, published April 30, 2025. Title: 靶向CD73的纳米抗体及纳米抗体-药物偶联物、其制备方法和用途. Applicant: 复旦大学. The sequence listing filed with the application follows.

SEQUENCE LISTING (56 sequences)

SEQ ID NO: 1 - protein, 8 aa, synthetic construct
  source 1..8: note = 3-D7 CDR1
GFLLDYYV

SEQ ID NO: 2 - protein, 8 aa, synthetic construct
  source 1..8: note = 3-D7 CDR2
ISGSDRST

SEQ ID NO: 3 - protein, 21 aa, synthetic construct
  source 1..21: note = 3-D7 CDR3
AADPSPVTVQAMCLPRFPVPY

SEQ ID NO: 4 - protein, 128 aa, synthetic construct
  source 1..128: note = 3-D7 VH
QRQLVESGGGLVQPGGSLRLSCAASGFLLDYYVIGWFRQAPGKEREGVSCISGSDRSTYYADSVKGRFTISRDNAKNTVYLQMNSLKPEDTAVYFCAADPSPVTVQAMCLPRFPVPYWGQGTQVTVST

SEQ ID NO: 5 - protein, 8 aa, synthetic construct
  source 1..8: note = 5-E11 CDR1
GFTLDYYN

SEQ ID NO: 6 - protein, 8 aa, synthetic construct
  source 1..8: note = 5-E11 CDR2
SSNSGGST

SEQ ID NO: 7 - protein, 17 aa, synthetic construct
  source 1..17: note = 5-E11 CDR3
AAYRGWHPSLDARVYDY

SEQ ID NO: 8 - protein, 124 aa, synthetic construct
  source 1..124: note = 5-E11 VH
ALQLVESGGGLVQPGGSLRLSCEVSGFTLDYYNIGWFRQAPGKEREGVSCSSNSGGSTYYADSVKGRFTISRDNAKNTVYLQMNSLKPEDTGVYYCAAYRGWHPSLDARVYDYWGQGTEVTVSS

SEQ ID NO: 9 - protein, 8 aa, synthetic construct
  source 1..8: note = 4-D04 CDR1
GFTLDYYN

SEQ ID NO: 10 - protein, 8 aa, synthetic construct
  source 1..8: note = 4-D04 CDR2
ISSSEGST

SEQ ID NO: 11 - protein, 17 aa, synthetic construct
  source 1..17: note = 4-D04 CDR3
AADRYYYCSLHVSQYDY

SEQ ID NO: 12 - protein, 124 aa, synthetic construct
  source 1..124: note = 4-D04 VH
QLQLVESGGGLVQPGGSLRLSCAASGFTLDYYNIGWFRQAPGKEREGVSCISSSEGSTYYADSVKGRFTISRDNAKNTVYLQMNSLKPEDTAVYYCAADRYYYCSLHVSQYDYWGQGTLVTVSS

SEQ ID NO: 13 - protein, 8 aa, synthetic construct
  source 1..8: note = 4-B02 CDR1
GFPLDYYS

SEQ ID NO: 14 - protein, 8 aa, synthetic construct
  source 1..8: note = 4-B02 CDR2
IGSSDGST

SEQ ID NO: 15 - protein, 17 aa, synthetic construct
  source 1..17: note = 4-B02 CDR3
AALKYYYCSGHEAIYDY

SEQ ID NO: 16 - protein, 124 aa, synthetic construct
  source 1..124: note = 4-B02 VH
EVQLVESGGGLVQPGGSLRLSCAASGFPLDYYSIGWFRQAPGKEREGVSCIGSSDGSTYYADSVKGRFTISRDNAENTVWLQMNSLKPEDTAVYYCAALKYYYCSGHEAIYDYWGQGTQVTVSG

SEQ ID NO: 17 - protein, 8 aa, synthetic construct
  source 1..8: note = 1-E7 CDR1
GFTLDYYN

SEQ ID NO: 18 - protein, 8 aa, synthetic construct
  source 1..8: note = 1-E7 CDR2
ISNSDGST

SEQ ID NO: 19 - protein, 17 aa, synthetic construct
  source 1..17: note = 1-E7 CDR3
AAYRGWHPSLDARVYDY

SEQ ID NO: 20 - protein, 124 aa, synthetic construct
  source 1..124: note = 1-E7 VH
QVQLVESGGGLVQPGGSLRLSCAASGFTLDYYNIGWFRQAPGKEREGVSCISNSDGSTYYADSVKGRFTISRDNAKNTVYLQMNSLKPEDTAVYYCAAYRGWHPSLDARVYDYWGQGTQVTVSS

SEQ ID NO: 21 - protein, 8 aa, synthetic construct
  source 1..8: note = 2-B10 CDR1
GFTLDDNA

SEQ ID NO: 22 - protein, 8 aa, synthetic construct
  source 1..8: note = 2-B10 CDR2
MRTSDGDT

SEQ ID NO: 23 - protein, 21 aa, synthetic construct
  source 1..21: note = 2-B10 CDR3
AAALGTYYSGFYYLAGDGMDY

SEQ ID NO: 24 - protein, 128 aa, synthetic construct
  source 1..128: note = 2-B10 VH
QLQLVESGGGLVQPGGSLRLSCAASGFTLDDNAIGWFRQAPGKEREGVACMRTSDGDTYYADSVKGRFTISRDNAKNTMYLQMNSLKPEDTAVYYCAAALGTYYSGFYYLAGDGMDYWGKGTLVTVSS

SEQ ID NO: 25 - protein, 8 aa, synthetic construct
  source 1..8: note = 2-G9 CDR1
GFLLDYYT

SEQ ID NO: 26 - protein, 8 aa, synthetic construct
  source 1..8: note = 2-G9 CDR2
ISSSDSSP

SEQ ID NO: 27 - protein, 9 aa, synthetic construct
  source 1..9: note = 2-G9 CDR3
ALRANVYDY

SEQ ID NO: 28 - protein, 124 aa, synthetic construct
  source 1..124: note = 2-G9 VH
QLQLVESGGGLVQPGGSLRLSCAASGFLLDYYTIGWFRQAPGKELEGVSCISSSDSSPYDADSVKGRFTMSRDNANNTVYLQMNSLKPEDTAVYYCAAQRYYYCALRANVYDYWGQGTQVTVST

SEQ ID NO: 29 - protein, 8 aa, synthetic construct
  source 1..8: note = 3-A3 CDR1
GFPLDYYT

SEQ ID NO: 30 - protein, 8 aa, synthetic construct
  source 1..8: note = 3-A3 CDR2
ISSSDSSP

SEQ ID NO: 31 - protein, 9 aa, synthetic construct
  source 1..9: note = 3-A3 CDR3
SLRANVYDY

SEQ ID NO: 32 - protein, 124 aa, synthetic construct
  source 1..124: note = 3-A3 VH
QVQLVESGGGSVQPGGSLRLSCAASGFPLDYYTIGWFRQAPGKELEGVSCISSSDSSPYDADSVKGRFTMSRDNANNTVYLQMNSLKPEDTAVYYCAAQRYYYCSLRANVYDYWGQGTQVTVSS

SEQ ID NO: 33 - protein, 8 aa, synthetic construct
  source 1..8: note = 3-F1 CDR1
GFTLDYYT

SEQ ID NO: 34 - protein, 8 aa, synthetic construct
  source 1..8: note = 3-F1 CDR2
IRSSDSSP

SEQ ID NO: 35 - protein, 9 aa, synthetic construct
  source 1..9: note = 3-F1 CDR3
SLTANVYDY

SEQ ID NO: 36 - protein, 124 aa, synthetic construct
  source 1..124: note = 3-F1 VH
QVQLVESGVSLVQPGGSLRLSCAASGFTLDYYTIGWFRQAPGKELEGISCIRSSDSSPYDADSVKDRFTMSRDNANNTVYLQMNSLKPEDTADYYCAAQRYYYCSLTANVYDYWGQGTQVTVSS

SEQ ID NO: 37 - protein, 360 aa, synthetic construct
  source 1..360: note = 3-D7-FC1
QRQLVESGGGLVQPGGSLRLSCAASGFLLDYYVIGWFRQAPGKEREGVSCISGSDRSTYYADSVKGRFTISRDNAKNTVYLQMNSLKPEDTAVYFCAADPSPVTVQAMCLPRFPVPYWGQGTQVTVSTEPKSSDKTHTCPPCPAPEFEGGPSVFLFPPKPKDTLMISRTPEVTCVVVDVSHEDPEVKFNWYVDGVEVHNAKTKPREEQYNSTYRVVSVLTVLHQDWLNGKEYKCKVSNKALPASIEKTISKAKGQPREPQVYTLPPSRDELTKNQVSLTCLVKGFYPSDIAVEWESNGQPENNYKTTPPVLDSDGSFFLYSKLTVDKSRWQQGNVFSCSVMHEALHNHYTQKSLSLSPGK

SEQ ID NO: 38 - protein, 364 aa, synthetic construct
  source 1..364: note = 3-D7-FC2
QRQLVESGGGLVQPGGSLRLSCAASGFLLDYYVIGWFRQAPGKEREGVSCISGSDRSTYYADSVKGRFTISRDNAKNTVYLQMNSLKPEDTAVYFCAADPSPVTVQAMCLPRFPVPYWGQGTQVTVSTGGGGSGGGGSGGGGSPCPAPEFEGGPSVFLFPPKPKDTLMISRTPEVTCVVVDVSHEDPEVKFNWYVDGVEVHNAKTKPREEQYNSTYRVVSVLTVLHQDWLNGKEYKCKVSNKALPASIEKTISKAKGQPREPQVYTLPPSRDELTKNQVSLTCLVKGFYPSDIAVEWESNGQPENNYKTTPPVLDSDGSFFLYSKLTVDKSRWQQGNVFSCSVMHEALHNHYTQKSLSLSPGKC

SEQ ID NO: 39 - protein, 361 aa, synthetic construct
  source 1..361: note = 3-D7-FC3
QRQLVESGGGLVQPGGSLRLSCAASGFLLDYYVIGWFRQAPGKEREGVSCISGSDRSTYYADSVKGRFTISRDNAKNTVYLQMNSLKPEDTAVYFCAADPSPVTVQAMCLPRFPVPYWGQGTQVTVSTEPKSSDKTHTCPPCPAPEFEGGPSVFLFPPKPKDTLMISRTPEVTCVVVDVSHEDPEVKFNWYVDGVEVHNAKTKPREEQYNSTYRVVSVLTVLHQDWLNGKEYKCKVSNKALPASIEKTISKAKGQPREPQVYTLPPSRDELTKNQVSLTCLVKGFYPSDIAVEWESNGQPENNYKTTPPVLDSDGSFFLYSKLTVDKSRWQQGNVFSCSVMHEALHNHYTQKSLSLSPGKC

SEQ ID NO: 40 - protein, 356 aa, synthetic construct
  source 1..356: note = 5E11-FC1
ALQLVESGGGLVQPGGSLRLSCEVSGFTLDYYNIGWFRQAPGKEREGVSCSSNSGGSTYYADSVKGRFTISRDNAKNTVYLQMNSLKPEDTGVYYCAAYRGWHPSLDARVYDYWGQGTEVTVSSEPKSSDKTHTCPPCPAPEFEGGPSVFLFPPKPKDTLMISRTPEVTCVVVDVSHEDPEVKFNWYVDGVEVHNAKTKPREEQYNSTYRVVSVLTVLHQDWLNGKEYKCKVSNKALPASIEKTISKAKGQPREPQVYTLPPSRDELTKNQVSLTCLVKGFYPSDIAVEWESNGQPENNYKTTPPVLDSDGSFFLYSKLTVDKSRWQQGNVFSCSVMHEALHNHYTQKSLSLSPGK

SEQ ID NO: 41 - protein, 360 aa, synthetic construct
  source 1..360: note = 5E11-FC2
ALQLVESGGGLVQPGGSLRLSCEVSGFTLDYYNIGWFRQAPGKEREGVSCSSNSGGSTYYADSVKGRFTISRDNAKNTVYLQMNSLKPEDTGVYYCAAYRGWHPSLDARVYDYWGQGTEVTVSSGGGGSGGGGSGGGGSPCPAPEFEGGPSVFLFPPKPKDTLMISRTPEVTCVVVDVSHEDPEVKFNWYVDGVEVHNAKTKPREEQYNSTYRVVSVLTVLHQDWLNGKEYKCKVSNKALPASIEKTISKAKGQPREPQVYTLPPSRDELTKNQVSLTCLVKGFYPSDIAVEWESNGQPENNYKTTPPVLDSDGSFFLYSKLTVDKSRWQQGNVFSCSVMHEALHNHYTQKSLSLSPGKC

SEQ ID NO: 42 - protein, 357 aa, synthetic construct
  source 1..357: note = 5E11-FC3
ALQLVESGGGLVQPGGSLRLSCEVSGFTLDYYNIGWFRQAPGKEREGVSCSSNSGGSTYYADSVKGRFTISRDNAKNTVYLQMNSLKPEDTGVYYCAAYRGWHPSLDARVYDYWGQGTEVTVSSEPKSSDKTHTCPPCPAPEFEGGPSVFLFPPKPKDTLMISRTPEVTCVVVDVSHEDPEVKFNWYVDGVEVHNAKTKPREEQYNSTYRVVSVLTVLHQDWLNGKEYKCKVSNKALPASIEKTISKAKGQPREPQVYTLPPSRDELTKNQVSLTCLVKGFYPSDIAVEWESNGQPENNYKTTPPVLDSDGSFFLYSKLTVDKSRWQQGNVFSCSVMHEALHNHYTQKSLSLSPGKC

SEQ ID NO: 43 - protein, 274 aa, synthetic construct
  source 1..274: note = 3-D7-HLE
QRQLVESGGGLVQPGGSLRLSCAASGFLLDYYVIGWFRQAPGKEREGVSCISGSDRSTYYADSVKGRFTISRDNAKNTVYLQMNSLKPEDTAVYFCAADPSPVTVQAMCLPRFPVPYWGQGTQVTVSTGGGGSGGGGCGGGGSEVQLVESGGGVVQPGGSLRLSCAASGLTFSSYAMGWFRQAPGKERERVVSISRGGGYTYYADSVKGRFTISRDNSENTVYLQMNSLRPEDTALYYCAAARYWATGSEYEFDYWGQGTLVTVSSAHHHHHHC

SEQ ID NO: 44 - protein, 207 aa, synthetic construct
  source 1..207: note = 3-D7-ABD
QRQLVESGGGLVQPGGSLRLSCAASGFLLDYYVIGWFRQAPGKEREGVSCISGSDRSTYYADSVKGRFTISRDNAKNTVYLQMNSLKPEDTAVYFCAADPSPVTVQAMCLPRFPVPYWGQGTQVTVSTGGGGSGGGGCGGGGSQHDEAVDANSLAEAKVLANRELDKYGVSDYYKNLINNAKTVEGVKALIDEILAALPAHHHHHHC

SEQ ID NO: 45 - protein, 203 aa, synthetic construct
  source 1..203: note = 5-E11-ABD
ALQLVESGGGLVQPGGSLRLSCEVSGFTLDYYNIGWFRQAPGKEREGVSCSSNSGGSTYYADSVKGRFTISRDNAKNTVYLQMNSLKPEDTGVYYCAAYRGWHPSLDARVYDYWGQGTEVTVSSGGGGSGGGGCGGGGSQHDEAVDANSLAEAKVLANRELDKYGVSDYYKNLINNAKTVEGVKALIDEILAALPAHHHHHHC

SEQ ID NO: 46 - protein, 124 aa, synthetic construct
  source 1..124: note = 5-E11 AS VH
ALQLVESGGGLVQPGGSLRLSCEVSGFTLDYYNIGWFRQAPGKEREGVSCSSASGGSTYYADSVKGRFTISRDNAKNTVYLQMNSLKPEDTGVYYCAAYRGWHPSLDARVYDYWGQGTEVTVSS

SEQ ID NO: 47 - protein, 124 aa, synthetic construct
  source 1..124: note = 5-E11 GS VH
ALQLVESGGGLVQPGGSLRLSCEVSGFTLDYYNIGWFRQAPGKEREGVSCSSGSGGSTYYADSVKGRFTISRDNAKNTVYLQMNSLKPEDTGVYYCAAYRGWHPSLDARVYDYWGQGTEVTVSS

SEQ ID NO: 48 - protein, 124 aa, synthetic construct
  source 1..124: note = 5-E11 QS VH
ALQLVESGGGLVQPGGSLRLSCEVSGFTLDYYNIGWFRQAPGKEREGVSCSSQSGGSTYYADSVKGRFTISRDNAKNTVYLQMNSLKPEDTGVYYCAAYRGWHPSLDARVYDYWGQGTEVTVSS

SEQ ID NO: 49 - protein, 124 aa, synthetic construct
  source 1..124: note = 5-E11 ASCS VH
ALQLVESGGGLVQPGGSLRLSCEVSGFTLDYYNIGWFRQAPGKEREGVSSSSASGGSTYYADSVKGRFTISRDNAKNTVYLQMNSLKPEDTGVYYCAAYRGWHPSLDARVYDYWGQGTEVTVSS

SEQ ID NO: 50 - protein, 128 aa, synthetic construct
  source 1..128: note = 3D7-HM7 VH
QRQLVESGGGLVQPGGSLRLSCAASGFLLDYYVIGWFRQAPGKEREGVSCISGSDRSTYYADSVKGRFTISRDNSKNTVYLQMGSLRAEDTAVYYCAADPSPVTVQAMCLPRFPVPYWGQGTLVTVSS

SEQ ID NO: 51 - protein, 128 aa, synthetic construct
  source 1..128: note = 3D7-HM8 VH
QRQLVESGGGLVQPGGSLRLSCAASGFLLDYYVIGWFRQAPGKEREGVSCISGSDRSTYYADSVKGRFTISRDNSKNTVYLQMSSLRAEDTAVYYCAADPSPVTVQAMCLPRFPVPYWGQGTLVTVSS

SEQ ID NO: 52 - protein, 128 aa, synthetic construct
  source 1..128: note = 3D7-HM9 VH
QRQLVESGGGLVQPGGSLRLSCAASGFLLDYYVIGWFRQAPGKEREGVSCISGSDRSTYYADSVKGRFTISRDNAKNTVYLQMSSLRAEDTAVYYCAADPSPVTVQAMCLPRFPVPYWGKGTLVTVSS

SEQ ID NO: 53 - protein, 212 aa, synthetic construct
  source 1..212: note = 3D7-HM9-ABD
QRQLVESGGGLVQPGGSLRLSCAASGFLLDYYVIGWFRQAPGKEREGVSCISGSDRSTYYADSVKGRFTISRDNAKNTVYLQMSSLRAEDTAVYYCAADPSPVTVQAMCLPRFPVPYWGKGTLVTVSSGGGGSGGGGSGGGGSQHDEAVDANSLAEAKVLANRELDKYGVSDYYKNLINNAKTVEGVKALIDEILAALPAAACAAAHHHHHH

SEQ ID NO: 54 - protein, 8 aa, synthetic construct
  source 1..8: note = 5-E11 AS CDR2 or 5-E11 ASCS CDR2
SSASGGST

SEQ ID NO: 55 - protein, 8 aa, synthetic construct
  source 1..8: note = 5-E11 GS CDR2
SSGSGGST

SEQ ID NO: 56 - protein, 8 aa, synthetic construct
  source 1..8: note = 5-E11 QS CDR2
SSQSGGST